European Patent Application EP 4 186 924 A1, published May 31, 2023. Title: Anti-Nipah Virus Monoclonal Antibody Having Neutralization Activity and Application. Applicant: ACADEMY OF MILITARY MEDICAL SCIENCE, PLA. Application CNPCT/2021/102585. The sequence listing filed with the application follows.

SEQUENCE LISTING (22 sequences)

SEQ ID NO: 1 - protein, 121 aa, Macaca mulatta
VQLQESGPGLVKPSETLSLTCAVSGDSISTGYDWTWIRQPPGKGLEWIGYIGGSSGNTNYNPSLKSRVTISKDTSKNQFSLKLSSVTAADTAVYYCARDGTRVYYYGLDSWGQGVVVTVSS

SEQ ID NO: 2 - DNA, 364 bp, Macaca mulatta
gtgcagctgcaggagtcgggcccagggctggtgaagccttcggagaccctgtccctcacctgcgctgtctctggtgactccatcagcactggttatgactggacctggatccgccagcccccagggaaagggctggagtggattgggtatatcggtggtagtagtggtaacaccaactacaatccctccctcaagagtcgagtcaccatttcaaaagacacgtccaagaaccagttctccctgaagctgagttctgtgaccgccgcggacaccgccgtgtattactgtgcgagagatggcacccgggtgtattactacggtttggattcctggggccaaggggtcgtcgtcaccgtctcctcag

SEQ ID NO: 3 - protein, 110 aa, Macaca mulatta
ETVVTQEPSLSVSPGGTVTLTCGLSSGSVSTSNYPSWFQQTPGQAPRMLIYSTNIRPSGVPNRFSGSILGNKAALTITGAQADDESDYYCFFSMVSGTSVFGGGTRLTVL

SEQ ID NO: 4 - DNA, 331 bp, Macaca mulatta
gagactgtggtgacccaggagccatcgttgtcagtgtcccctggaggaacagtcacactcacctgtggcctgagctctggctcagtctctaccagcaactaccccagctggttccagcagaccccaggccaggctccacgcatgctcatctacagtacaaatattcgcccttctggggtccctaatcgcttctctggctccatccttgggaacaaagctgccctcaccatcacgggggctcaggcagacgatgaatctgattactactgtttcttctccatggttagtggcacttcggttttcggcggagggacccggctgaccgtcctag

SEQ ID NO: 5 - protein, 116 aa, Macaca mulatta
EVQLVESGGGLVQPGGSLRLSCAASGFTFSSYDMSWVRQAPGKGLEWVSSISSVTSYISYADSVKGRFTISRDNAKNSLSLQMNSLKTEDTAVYYCTTENWNFDFWGQGVLVTVSS

SEQ ID NO: 6 - DNA, 349 bp, Macaca mulatta
gaggtgcaactggtggagtctgggggaggcttggtccagcctggagggtccctgagactctcctgtgcagcctctggattcaccttcagtagttacgacatgagctgggtccgccaggctccgggaaaggggctggagtgggtctcatccattagtagtgttactagttacatatcctacgctgactccgtgaagggccgattcaccatctccagagacaacgccaagaactcgctgtctctgcaaatgaacagcctgaaaaccgaggacacggccgtatattactgtactactgaaaactggaactttgacttctggggccagggagtcctggtcaccgtctcctcag

SEQ ID NO: 7 - protein, 113 aa, Macaca mulatta
DVVMTQSPLSLATTPGQPASISCRSSQSLVHSNGNTYLSWYQQKPGQPPRLLIYEVSNRDSGVPDRFSGSGAGTDFTLKISRVEAEDVGVYYCGQGTHWPPFTFGPGTKLDIK

SEQ ID NO: 8 - DNA, 340 bp, Macaca mulatta
gatgttgtgatgactcagtctccactctccctggccaccacccctggacagccggcctccatctcctgcaggtctagtcaaagccttgtacacagtaatggaaacacctacttgagttggtatcagcagaagccaggccaacctccaaggctcctgatttatgaggtttctaaccgggactctggggtcccagacagattcagcggcagtggggcagggacagatttcacactgaaaatcagcagagtggaggctgaggatgttggggtttattactgcgggcaaggtacacactggcctccgttcactttcggccccgggaccaaactggatatcaaac

SEQ ID NO: 9 - protein, 121 aa, Macaca mulatta
QVQLQESGPGLVKPSETLSLSCAVSGGSFSDYWWGWIRQSPGKGLEWIGSIYGSSGRTAYSPSLKSRATISRDTSKNQLFLRLTSVTAADTGVYYCTNERFYGDSNRFDVWGPGVLVTVSS

SEQ ID NO: 10 - DNA, 364 bp, Macaca mulatta
caggtgcagctgcaggagtcgggcccaggactggtgaagccttcggagaccctgtccctctcctgcgctgtctctggtggctccttcagcgattactggtggggctggatccgccagtccccagggaaggggctggagtggattgggagtatctatggtagtagtgggcgaaccgcatacagcccctccctcaaaagtcgagccaccatttcaagagacacgtccaagaaccagctcttcctgaggctgacctctgtgaccgccgcggacacgggagtctactactgtaccaacgagaggttctacggtgacagcaaccggttcgatgtctggggcccgggagtcctggtcaccgtctcctcag

SEQ ID NO: 11 - protein, 115 aa, Macaca mulatta
QPVLTQPTSLSASPGASARLTCTLSSGISVGNYRIFWYQQKPGSPPRYLLNYHTDSDKHQGSGVPSRFSGSKDASANAGILLISGLQSEDEADYYCMIWHNNVDVFGGGTKLTVL

SEQ ID NO: 12 - DNA, 346 bp, Macaca mulatta
cagcctgtgctgactcagccaacctccctctcagcatctcctggagcatcagccagactcacctgcaccttgagcagtggcatcagtgttggtaattacaggattttctggtaccagcagaagccagggagtcctccccggtatcttctgaactaccacacagactcagataagcaccagggctctggagtccccagtcgcttctctggatccaaagatgcttcggccaatgcagggattttactcatctctgggctccagtctgaggatgaggctgactattactgtatgatttggcacaacaatgttgatgtgttcggaggtggcaccaagttgaccgtcctcg

SEQ ID NO: 13 - protein, 119 aa, Macaca mulatta
QVQLVQSGAEVKKPGASVKLSCKASGYTFTSFYINWVRQAPGQVLEWMGWINPSNGDTGYAQKFQGRVTMSRDTSTSTAYMELSSLRSEDTAVYYCTRETVGSGTFDCWGQGVLVTVSS

SEQ ID NO: 14 - DNA, 358 bp, Macaca mulatta
caggtccagctggtgcagtccggggctgaggtgaagaagcctggggcctcagtgaaactctcctgcaaggcttctggttacacctttaccagcttctatataaactgggtgagacaggcccctggacaagtgcttgagtggatgggatggattaaccctagcaatggtgatacaggctacgcacagaaattccagggcagagtcaccatgtccagggacacgtcgacgagtacagcctacatggagctgagcagcctgagatctgaggacacggccgtgtattattgtacgagagagactgttggtagtggaacctttgactgctggggccagggagtcctggtcaccgtctcctcag

SEQ ID NO: 15 - protein, 112 aa, Macaca mulatta
DIVMTQTPLSLSVTLGEPASISCRSSQSLVYSAGKTYLDWYLQKPGQSPQLLIYLVSKRASGVPDKFSGSGSGTDFTLKISRVEAEDVGVYYCMQALRSPLTFGGGTKVELK

SEQ ID NO: 16 - DNA, 337 bp, Macaca mulatta
gatattgtgatgacccagactccactctccctgtccgtcacccttggagagccggcctccatctcctgcaggtctagtcagagccttgtatacagtgctggaaaaacctatttggattggtacctgcagaagccaggccagtctccacagctcctaatatatttggtttccaaacgggcctctggagtcccagacaagttcagtggcagtgggtcaggcactgatttcacactgaaaatcagcagggtggaggctgaggatgttggggtttattactgcatgcaagctctacggtctccgctcactttcggcggagggaccaaggtggagctcaaac

SEQ ID NO: 17 - protein, 330 aa, Homo sapiens [sequence omitted]

SEQ ID NO: 18 - DNA, 990 bp, Homo sapiens
gcctccaccaagggcccatcggtcttccccctggcaccctcctccaagagcacctctgggggcacagcagccctgggctgcctggtcaaggactacttccccgaaccggtgacggtgtcgtggaactcaggcgccctgaccagcggcgtgcacaccttcccggctgtcctacagtcctcaggactctactccctcagcagcgtggtgaccgtgccctccagcagcttgggcacccagacctacatctgcaacgtgaatcacaagcccagcaacaccaaggtggacaagaaagttgagcccaaatcttgtgacaaaactcacacatgcccaccgtgcccagcacctgaactcctggggggaccgtcagtcttcctcttccccccaaaacccaaggacaccctcatgatctcccggacccctgaggtcacatgcgtggtggtggacgtgagccacgaagaccctgaggtcaagttcaactggtacgtggacggcgtggaggtgcataatgccaagacaaagccgcgggaggagcagtacaacagcacgtaccgtgtggtcagcgtcctcaccgtcctgcaccaggactggctgaatggcaaggagtacaagtgcaaggtctccaacaaagccctcccagcccccatcgagaaaaccatctccaaagccaaagggcagccccgagaaccacaggtgtacaccctgcccccatcccgggatgagctgaccaagaaccaggtcagcctgacctgcctggtcaaaggcttctatcccagcgacatcgccgtggagtgggagagcaatgggcagccggagaacaactacaagaccacgcctcccgtgctggactccgacggctccttcttcctctacagcaagctcaccgtggacaagagcaggtggcagcaggggaacgtcttctcatgctccgtgatgcatgaggctctgcacaaccactacacacagaagagcctctccctgtctccgggtaaa

SEQ ID NO: 19 - protein, 106 aa, Homo sapiens
TVAAPSVFIFPPSDEQLKSGTASVVCLLNNFYPREAKVQWKVDNALQSGNSQESVTEQDSKDSTYSLSSTLTLSKADYEKHKVYACEVTHQGLSSPVTKSFNRGEC

SEQ ID NO: 20 - DNA, 318 bp, Homo sapiens
actgtggctgcaccatctgtcttcatcttcccgccatctgatgagcagttgaaatctggaactgcctctgttgtgtgcctgctgaataacttctatcccagagaggccaaagtacagtggaaggtggataacgccctccaatcgggtaactcccaggagagtgtcacagagcaggacagcaaggacagcacctacagcctcagcagcaccctgacgctgagcaaagcagactacgagaaacacaaagtctacgcctgcgaagtcacccatcagggcctgagttcgcccgtcacaaagagcttcaacaggggagagtgt

SEQ ID NO: 21 - protein, 106 aa, Homo sapiens [sequence omitted]

SEQ ID NO: 22 - DNA, 318 bp, Homo sapiens
cgtcagcccaaggctgccccctcggtcactctgttcccaccctcgagtgaggagcttcaagccaacaaggccacactggtgtgtctcataagtgacttctacccgggagccgtgacagtggcctggaaggcagatagcagccccgtcaaggcgggagtggagaccaccacaccctccaaacaaagcaacaacaagtacgcggccagcagctacctgagcctgacgcctgagcagtggaagtcccacaaaagctacagctgccaggtcacgcatgaagggagcaccgtggagaagacagtggcccctacagaatgttca